European Patent Specification EP 3 710 043 B1, published April 17, 2024. Title: METHOD FOR THE TREATMENT OF HEART DISEASES. Applicant: UNIVERSITE D'AIX-MARSEILLE et al. The sequence listing filed with the application follows.

SEQUENCE LISTING (38 sequences)

SEQ ID NO: 1 - DNA, 27 bp, artificial
  primer
cttccagtatgttccttctgatgagac

SEQ ID NO: 2 - DNA, 25 bp, artificial
  primer
tacggacagtcttcttcttggtccc

SEQ ID NO: 3 - DNA, 30 bp, artificial
  primer
gagcttgctgggggaaacttcctgactagg

SEQ ID NO: 4 - DNA, 20 bp, artificial
  primer
atcctctgcatggtcaggtc

SEQ ID NO: 5 - DNA, 18 bp, artificial
  primer
cgtggcctgattcattcc

SEQ ID NO: 6 - DNA, 23 bp, artificial
  primer
aagtcgctctgagttgttatcag

SEQ ID NO: 7 - DNA, 22 bp, artificial
  primer
ggagcgggagaaatggatatga

SEQ ID NO: 8 - DNA, 24 bp, artificial
  primer
cgggttgttaaaccttcgattccg

SEQ ID NO: 9 - DNA, 17 bp, artificial
  primer
gacgccatccacgctgt

SEQ ID NO: 10 - DNA, 20 bp, artificial
  primer
tgctgccagttaaaagatgc

SEQ ID NO: 11 - DNA, 23 bp, artificial
  primer
caacacagatctgatggatttca

SEQ ID NO: 12 - DNA, 20 bp, artificial
  primer
cctcatcttctaccggcatc

SEQ ID NO: 13 - DNA, 21 bp, artificial
  primer
gtcagtcgtttgggctgtaac

SEQ ID NO: 14 - DNA, 20 bp, artificial
  primer
agacccaggcagagtcagaa

SEQ ID NO: 15 - DNA, 21 bp, artificial
  primer
catgttcagctttgtggacct

SEQ ID NO: 16 - DNA, 20 bp, artificial
  primer
gcagctgacttcagggatgt

SEQ ID NO: 17 - DNA, 19 bp, artificial
  primer
tggtcctgctggaaaggat

SEQ ID NO: 18 - DNA, 18 bp, artificial
  primer
gaggtccaggcagtccac

SEQ ID NO: 19 - DNA, 20 bp, artificial
  primer
gagaagaacggcaaggtcag

SEQ ID NO: 20 - DNA, 20 bp, artificial
  primer
tttccccttcttgttcatgg

SEQ ID NO: 21 - DNA, 20 bp, artificial
  primer
ctggtgaaaaggacctctcg

SEQ ID NO: 22 - DNA, 20 bp, artificial
  primer
tggcaacatcaacaggactc

SEQ ID NO: 23 - DNA, 20 bp, artificial
  primer
aactaacccgggacttggag

SEQ ID NO: 24 - DNA, 20 bp, artificial
  primer
agtagaactcgggcaagctg

SEQ ID NO: 25 - DNA, 20 bp, artificial
  primer
cctcaagctcatggctacac

SEQ ID NO: 26 - DNA, 20 bp, artificial
  primer
ttgcctcctttgcctttacc

SEQ ID NO: 27 - DNA, 20 bp, artificial
  primer
aggcaaagaaaggctcatcc

SEQ ID NO: 28 - DNA, 20 bp, artificial
  primer
tggagcgcaagtttgtcata

SEQ ID NO: 29 - DNA, 21 bp, artificial
  primer
agcctcttctcattcctgctt

SEQ ID NO: 30 - DNA, 19 bp, artificial
  primer
atgagagggaggccatttg

SEQ ID NO: 31 - DNA, 20 bp, artificial
  primer
ctcgctcagcaccttctctc

SEQ ID NO: 32 - DNA, 19 bp, artificial
  primer
cactctgggtggctgagtc

SEQ ID NO: 33 - DNA, 20 bp, artificial
  primer
gaaggagaactgcccgtaca

SEQ ID NO: 34 - DNA, 22 bp, artificial
  primer
ggcaacaactccgatttctact

SEQ ID NO: 35 - DNA, 20 bp, artificial
  primer
atgctggacccaacacaaat

SEQ ID NO: 36 - DNA, 21 bp, artificial
  primer
tctttcactttgccaaacacc

SEQ ID NO: 37 - DNA, 20 bp, artificial
  primer
gtggacatcggatacccaag

SEQ ID NO: 38 - DNA, 20 bp, artificial
  primer
aagttggaaggccggttaat